European Patent Application EP 4 212 549 A1, published July 19, 2023. Title: 一组GITR单克隆抗体及其医药用途. Applicant: 东大生物技术（苏州）有限公司. The sequence listing filed with the application follows.

SEQUENCE LISTING (131 sequences)

SEQ ID NO: 1 - protein, 118 aa, 鼠
  4E1
DVQLQESGPGLVKPSQSLSLTCTVTGYSITSDYAWNWIRQFPGNKLEWMGYIRNSGTTSYNPSLKSRISITRDTSKNHFFLQLNSVTTEDTATYYCTRSGHHDLFDYWGQGTTLTVSS

SEQ ID NO: 2 - protein, 6 aa, 人工
  4E1
SDYAWN

SEQ ID NO: 3 - protein, 16 aa, 人工
  4E1
YIRNSGTTSYNPSLKS

SEQ ID NO: 4 - protein, 9 aa, 人工
  4E1
SGHHDLFDY

SEQ ID NO: 5 - protein, 114 aa, 鼠
  4E1
DVVMTQTPLTLSFTIGQPASISCKSSQSLLDSDGKTYLNWLLQRPGQSPKRLIYLVSELDSGVPDRFTGSGSGTDFTLQISRVEAEDLGVYYCWQGTHFPWTFGGGTKLEIKRA

SEQ ID NO: 6 - protein, 16 aa, 人工
  4E1
KSSQSLLDSDGKTYLN

SEQ ID NO: 7 - protein, 7 aa, 人工
  4E1
LVSELDS

SEQ ID NO: 8 - protein, 9 aa, 人工
  4E1
WQGTHFPWT

SEQ ID NO: 9 - protein, 116 aa, 鼠
  8H4
EVQLQQSGPELVRPGASVNISCKASGYTFTDYYMNWVKQSHGKSLEWIGNINPNHDYTSYNQKFKGKATLTVDKSSNTAYMELRSLTSEDSAVYYCARYYYAMDYWGQGTSVTVSS

SEQ ID NO: 10 - protein, 5 aa, 人工
  8H4
DYYMN

SEQ ID NO: 11 - protein, 17 aa, 人工
  8H4
NINPNHDYTSYNQKFKG

SEQ ID NO: 12 - protein, 7 aa, 人工
  8H4
YYYAMDY

SEQ ID NO: 13 - protein, 108 aa, 鼠
  8H4
QIVLTQSPAIMSAFPGEKVTMTCSASSSVSYMYWYQQKPGSSPRLLIFDTSTLASGVPVRFSGSGSGTSHSLTISRMEAEDAATYYCQQWSSFPPTFGAGTRLELKRA

SEQ ID NO: 14 - protein, 10 aa, 人工
  8H4
SASSSVSYMY

SEQ ID NO: 15 - protein, 7 aa, 人工
  8H4
DTSTLAS

SEQ ID NO: 16 - protein, 9 aa, 人工
  8H4
QQWSSFPPT

SEQ ID NO: 17 - protein, 115 aa, 鼠
  4E4
EVQLQQSGPELVKPGASVKISCKASGYTFTDHYMNWVKQSHGKSLEWIGDIDPKNGGTLYNQNFKGRATLTVDKSSSTAYMDLRSLTSEDSAVYYCARREAMDYWGQGTSVTVSS

SEQ ID NO: 18 - protein, 5 aa, 人工
  4E4
DHYMN

SEQ ID NO: 19 - protein, 17 aa, 人工
  4E4
DIDPKNGGTLYNQNFKG

SEQ ID NO: 20 - protein, 6 aa, 人工
  4E4
REAMDY

SEQ ID NO: 21 - protein, 114 aa, 鼠
  4E4
DVLMTQIPLSLPVSFGDQASISCRSSQSIVYSNGNTYLNWYLQKPGQSPKLLIYKVSNRFSGVPDRFSGSGSGTDFTLKISRVEAEDLGVYYCFQGSHVPWTFGGGTKLEIKRA

SEQ ID NO: 22 - protein, 16 aa, 人工
  4E4
RSSQSIVYSNGNTYLN

SEQ ID NO: 23 - protein, 7 aa, 人工
  4E4
KVSNRFS

SEQ ID NO: 24 - protein, 9 aa, 人工
  4E4
FQGSHVPWT

SEQ ID NO: 25 - protein, 116 aa, 鼠
  3F5
EVQLQQSGPELVKPGTSVKISCKASGYTFTDHYMHWVRQSHGKSLEWIGDINPNSGGTINNQNFKGKATLTVDKSSNTAYMGLHSLTSEDSAVYYCASGFSGLAYWGQGTLVTVSA

SEQ ID NO: 26 - protein, 6 aa, 人工
  3F5
SDYAWN

SEQ ID NO: 27 - protein, 16 aa, 人工
  3F5
YIRNSGTTSYNPSLKS

SEQ ID NO: 28 - protein, 9 aa, 人工
  3F5
SGHHDLFDY

SEQ ID NO: 29 - protein, 114 aa, 鼠
  3F5
DVVMTQTPLTLSVTIGQPASISCKSSQSLLDRDGKTYLNWLFQRPGQSLKRLIYLVSILDSGVPDRFTGSGSGTDFTLKISRVEAGDLGIYYCWQGTHFPWTFGGGTKLEIKRA

SEQ ID NO: 30 - protein, 16 aa, 人工
  3F5
KSSQSLLDRDGKTYLN

SEQ ID NO: 31 - protein, 7 aa, 人工
  3F5
LVSILDS

SEQ ID NO: 32 - protein, 7 aa, 人工
  3F5
LVSILDS

SEQ ID NO: 33 - protein, 117 aa, 鼠
  4C1
QVQLQQSGAELARPGASVKLSCKASGYTFTSYWMQWVKQRPGQGLEWIGTIYPGDGDTRYTQKFKGKATLTADKSSNTAYMQLSSLASEDSAVYYCARFEGRQFAYWGQGTLVTVSA

SEQ ID NO: 34 - protein, 5 aa, 人工
  4C1
DHYMH

SEQ ID NO: 35 - protein, 17 aa, 人工
  4C1
DINPNSGGTINNQNFKG

SEQ ID NO: 36 - protein, 7 aa, 人工
  4C1
GFSGLAY

SEQ ID NO: 37 - protein, 106 aa, 鼠
  4C1
MTQSPASLSVSVGETVTITCRASENIYSNLAWYQQKQGKSPQLLVYAATNLADGVPSRFSGSGSGTQYSLKINSLQSEDFGSYYCQHFWGPPWTFGGGTKLEIKRA

SEQ ID NO: 38 - protein, 11 aa, 人工
  4C1
RASENIYSNLA

SEQ ID NO: 39 - protein, 7 aa, 人工
  4C1
AATNLAD

SEQ ID NO: 40 - protein, 9 aa, 人工
  4C1
QHFWGPPWT

SEQ ID NO: 41 - protein, 118 aa, 鼠
  7D7
QVQLQQSGAEVMKPGASVKISCKATDYIFSRYWIEWVKQRPGHGLEWIGEILPGSGYNNSNDKFKGKATFTADTSSNTAYMQLSSLTFEDSAVYYCARKGTFYTMDHWGQGTSVTVSS

SEQ ID NO: 42 - protein, 5 aa, 人工
  7D7
NYLIE

SEQ ID NO: 43 - protein, 17 aa, 人工
  7D7
VINPGSGNTNYNEKFKG

SEQ ID NO: 44 - protein, 14 aa, 人工
  7D7
GYYGYSRNYYAMDY

SEQ ID NO: 45 - protein, 110 aa, 鼠
  7D7
DIVMTQSTAIMSASLGERVTMTCTASSSVSSSYFHWYQQKPGSSPKLWIYSTSNLASGVPARFSGRGSGTSYSLTISSVEAEDAATYYCHQYHHSPRTFGGGSKLEIKRA

SEQ ID NO: 46 - protein, 12 aa, 人工
  7D7
TASSSVSSSYFH

SEQ ID NO: 47 - protein, 7 aa, 人工
  7D7
STSNLAS

SEQ ID NO: 48 - protein, 9 aa, 人工
  7D7
HQYHHSPRT

SEQ ID NO: 49 - protein, 117 aa, 鼠
  7E11
QVQLQQSGAELARPGASVKLSCKASGYTFTSYWMQWIKQRPGQGLEWIGTIYPGDGDTRYTQKFKGKATLTADKSSSTAYMQLSSLASEDSAVYYCARFEGRQFAYWGQGTLVTVSA

SEQ ID NO: 50 - protein, 5 aa, 人工
  7E11
NYAMV

SEQ ID NO: 51 - protein, 17 aa, 人工
  7E11
YINPTSGYSKYNQSFRD

SEQ ID NO: 52 - protein, 9 aa, 人工
  7E11
SPLLGNLDY

SEQ ID NO: 53 - protein, 109 aa, 鼠
  7E11
DIQMTQSPASLSVSVGETVTITCRASENIYSNLAWYQQKQGKSPQLLVYAATNLADGVPSRFSGSGSGTQYSLKINSLQSEDFGSYYCQHFWGPPWTFGGGTKLEIKRA

SEQ ID NO: 54 - protein, 11 aa, 人工
  7E11
RASENIYSNLA

SEQ ID NO: 55 - protein, 7 aa, 人工
  7E11
AATNLAD

SEQ ID NO: 56 - protein, 9 aa, 人工
  7E11
QHFWGPPWT

SEQ ID NO: 57 - protein, 118 aa, 鼠
  10E11
EVKLEESGGGLVNLGASVKISCKATGYPVSRYWIEWLKQRPGHGPEWIGEILPGSDYANYNEKFKGKATFTADISSNSAYMQLSSLTSEDSAVYYCSRKGAYYALDFWGQGTSVTVSS

SEQ ID NO: 58 - protein, 5 aa, 人工
  10E11
RYWIE

SEQ ID NO: 59 - protein, 17 aa, 人工
  10E11
EILPGSDYANYNEKFKG

SEQ ID NO: 60 - protein, 9 aa, 人工
  10E11
KGAYYALDF

SEQ ID NO: 61 - protein, 109 aa, 鼠
  10E11
DIVLTQSPATLSVTPGERVSLSCRASQSVNNYLHWYQQKSHESPRLLISYASQSISGISSRFSGSGSGTDFTLIIHSVETEDFGMYFCQQSNRWPLTFGAGTKLELKRA

SEQ ID NO: 62 - protein, 11 aa, 人工
  10E11
RASQSVNNYLH

SEQ ID NO: 63 - protein, 7 aa, 人工
  10E11
YASQSIS

SEQ ID NO: 64 - protein, 9 aa, 人工
  10E11
QQSNRWPLT

SEQ ID NO: 65 - protein, 117 aa, 鼠
  3G12
QVQLQQSGAELARPGASVKLSCKASGYTFTSYWMQWVKQRPGQGLEWIGTIYPGDGDTRYTQKFKGKATLTADKSSSTVYMQLTSLASEDSAVYYCARFYGGAMDSWGQGTSVTVSS

SEQ ID NO: 66 - protein, 5 aa, 人工
  3G12
RYWIE

SEQ ID NO: 67 - protein, 17 aa, 人工
  3G12
EILPGSGYNNSNDKFKG

SEQ ID NO: 68 - protein, 9 aa, 人工
  3G12
KGTFYTMDH

SEQ ID NO: 69 - protein, 109 aa, 鼠
  3G12
DIQMTQSPASLSVSVGETVTITCRASENIYSNLAWYQHKQGKSPQLLVYAATNLADGVPSRFSGGGSGTQYSLKINSLQSEDFGTYYCQHFWGPPWTFGGGTKLEIKRA

SEQ ID NO: 70 - protein, 11 aa, 人工
  3G12
RASENIYSNLA

SEQ ID NO: 71 - protein, 7 aa, 人工
  3G12
AATNLAD

SEQ ID NO: 72 - protein, 9 aa, 人工
  3G12
QHFWGPPWT

SEQ ID NO: 73 - protein, 119 aa, 鼠
  4B11
EVQLQQSGPELVKPGASVKMSCKASGFTFTDSVLHWVKQKPGQGLEWIGYIHPYNDDTKFHDSFKGKATLTSDKSSTTAYMELSSLTSEDSAVYYCSRNDELRVALDYWGQGTSVTVSS

SEQ ID NO: 74 - protein, 5 aa, 人工
  4B11
SYWMQ

SEQ ID NO: 75 - protein, 17 aa, 人工
  4B11
TIYPGDGDTRYTQKFKG

SEQ ID NO: 76 - protein, 8 aa, 人工
  4B11
FEGRQFAY

SEQ ID NO: 77 - protein, 113 aa, 鼠
  4B11
DIVLTQSPASLAVSLGQRATISCRASQSVSTSTYSYVHWYQQKPGQPPKLLIKYASNLESGVPARFSGRGSGTDFTLSIHPVEGEDAATYYCQHSWGNPWTFGGGTKLEIKRA

SEQ ID NO: 78 - protein, 15 aa, 人工
  4B11
RASQSVSTSTYSYVH

SEQ ID NO: 79 - protein, 7 aa, 人工
  4B11
YASNLES

SEQ ID NO: 80 - protein, 9 aa, 人工
  4B11
QHSWGNPWT

SEQ ID NO: 81 - protein, 115 aa, 鼠
  5F1
DVQLQESGPGLVKPSHSLSLTCTVTGYSITSDYAWNWIRQFPGNNLEWMGYITYSGSTGYNPSLKSRISITRDTSKNQFFLQLNSVTAEDTATYYCARDWPFAYWGQGTLVTVSA

SEQ ID NO: 82 - protein, 5 aa, 人工
  5F1
RYWIE

SEQ ID NO: 83 - protein, 17 aa, 人工
  5F1
EILPGSDYANYNEKFKG

SEQ ID NO: 84 - protein, 9 aa, 人工
  5F1
KGAYYALDF

SEQ ID NO: 85 - protein, 108 aa, 鼠
  5F1
QIVLTQSPAIMSASPGEKATITCSASSSVSYMHWFQQRPGTSPKLWIYSTSNLASGVPARFSGSGSGTSFSLTISRMEAEDAATYYCHQRSGHTFTFGSGTKLEIKRA

SEQ ID NO: 86 - protein, 10 aa, 人工
  5F1
SASSSVSYMH

SEQ ID NO: 87 - protein, 7 aa, 人工
  5F1
STSNLAS

SEQ ID NO: 88 - protein, 9 aa, 人工
  5F1
HQRSGHTFT

SEQ ID NO: 89 - protein, 119 aa, 鼠
  5F6
EVKLEESGGGLVQPGGSLKLSCAASGFTLSRYTMSWVRQTPEKRLEWVAYISNGGGSTYYPDTVKGRFTTSRDNAKNTLYLQMSSLKSEDTAMYYCGRAEAGTDWFAYWGQGTLVTVSA

SEQ ID NO: 90 - protein, 5 aa, 人工
  5F6
SYWMQ

SEQ ID NO: 91 - protein, 17 aa, 人工
  5F6
TIYPGDGDTRYTQKFKG

SEQ ID NO: 92 - protein, 8 aa, 人工
  5F6
FYGGAMDS

SEQ ID NO: 93 - protein, 113 aa, 鼠
DIVLTQSPASLAVSLGQRATISCRASQSVSTSSYSYMHWYQQKPGQPPKLLIKYASNLESGVPARFSGSGSGTDFTLNIHPVEEEDTATYYCQHGWEIPYTFGGGTKLEIKRA

SEQ ID NO: 94 - protein, 15 aa, 人工
  5F6
RASQSVSTSSYSYMH

SEQ ID NO: 95 - protein, 7 aa, 人工
  5F6
YASNLES

SEQ ID NO: 96 - protein, 9 aa, 人工
  5F6
QHGWEIPYT

SEQ ID NO: 97 - protein, 119 aa, 鼠
  13G12
QVQLQQPGTELVKPGASVKLSCKASGYTFTSNWMNWVKQRPGHGLEWIGNIYPSNGGTNYNEKFKSKATLTVDKSSSTAYMQLRGLTSEDSAVYYCVRHSNYVGAMDYWGQGTSVTVSS

SEQ ID NO: 98 - protein, 5 aa, 人工
  13G12
DSVLH

SEQ ID NO: 99 - protein, 17 aa, 人工
  13G12
YIHPYNDDTKFHDSFKG

SEQ ID NO: 100 - protein, 10 aa, 人工
  13G12
NDELRVALDY

SEQ ID NO: 101 - protein, 108 aa, 鼠
  13G12
QIVLTQSPAIMSASPGEKVTMTCGASSSVSYMYWFQQKPGSSPRLLIYDTFNLASGVPVRFSGSESGTSYSLTISRMEAEDAATYYCQHWSSYPPTFGSGTKLEIDRA

SEQ ID NO: 102 - protein, 10 aa, 人工
  13G12
GASSSVSYMY

SEQ ID NO: 103 - protein, 7 aa, 人工
  13G12
DTFNLAS

SEQ ID NO: 104 - protein, 9 aa, 人工
  13G12
QHWSSYPPT

SEQ ID NO: 105 - protein, 118 aa, 鼠
  9B3
QVQLQQSGAELMNLGASVKISCKATGYPVSRYWIEWLKQRPGHGPEWIGEILPGSDYANYNEKFKGKATFTADISSNSAYMQLSSLTSEDSAVYYCSRKGAYYALDFWGQGTSVTVSS

SEQ ID NO: 106 - protein, 6 aa, 人工
  9B3
SDYAWN

SEQ ID NO: 107 - protein, 16 aa, 人工
  9B3
YITYSGSTGYNPSLKS

SEQ ID NO: 108 - protein, 6 aa, 人工
  9B3
DWPFAY

SEQ ID NO: 109 - protein, 107 aa, 鼠
  9B3
DIVMTQSPATLSVTPGERVSLSCRASQSVNNYLHWYQQKSHESPRLLISYVSQSISGISSRFSGSGSGTDFTLIIHSVETEDFGMYFCQQSNRWPLTFGAGTKLELK

SEQ ID NO: 110 - protein, 11 aa, 人工
  9B3
RASQSVNNYLH

SEQ ID NO: 111 - protein, 7 aa, 人工
  9B3
YVSQSIS

SEQ ID NO: 112 - protein, 9 aa, 人工
  9B3
QQSNRWPLT

SEQ ID NO: 113 - protein, 115 aa, 人源化
  4E4
QVQLVQSGAEVKKPGASVKVSCKASGYTFTDHYMNWVRQAPGQGLEWIGDIDPKNGGTLYNQNFKGRATLTVDKSISTAYMELSRLRSDDTAVYYCARREAMDYWGQGTLVTVSS

SEQ ID NO: 114 - protein, 112 aa, 人源化
  4E4
DVVMTQSPLSLPVTPGEPASISCRSSQSIVYSNGNTYLNWYLQKPGQSPQLLIYKVSNRFSGVPDRFSGSGSGTDFTLKISRVEAEDVGVYYCFQGSHVPWTFGGGTKVEIK

SEQ ID NO: 115 - protein, 119 aa, 人源化
  4B11
EVQLVQSGAEVKKPGASVKVSCKASGFTFTDSVLHWVRQAPGQRLEWIGYIHPYNDDTKFHDSFKGRATLTSDKSASTAYMELSSLRSEDTAVYYCSRNDELRVALDYWGQGTLVTVSS

SEQ ID NO: 116 - protein, 111 aa, 人源化
  4B11
EIVLTQSPATLSLSPGERATLSCRASQSVSTSTYSYVHWYQQKPGQAPRLLIKYASNLESGIPARFSGSGSGTDFTLTISSLEPEDFAVYYCQHSWGNPWTFGGGTKVEIK

SEQ ID NO: 117 - protein, 116 aa, 人源化
  3F5
QVQLVQSGAEVKKPGASVKVSCKASGYTFTDHYMHWVRQAPGQGLEWIGDINPNSGGTINNQNFKGRATLTVDKSISTAYMELSRLRSDDTAVYYCARGFSGLAYWGQGTLVTVSS

SEQ ID NO: 118 - protein, 112 aa, 人源化
  3F5
DIVMTQTPLSSPVTLGQPASISCKSSQSLLDRDGKTYLNWLQQRPGQPPRRLIYLVSILDSGVPDRFSGSGAGTDFTLKISRVEAEDVGVYYCWQGTHFPWTFGQGTKLEIK

SEQ ID NO: 119 - protein, 118 aa, 人源化
  10E11
EVQLVQSGAEVKKPGESLRISCKGSGYPVSRYWIEWVRQMPGKGLEWIGEILPGSDYANYNEKFKGHATFSADISISTAYLQWSSLKASDTAMYYCSRKGAYYALDFWGQGTLVTVSS

SEQ ID NO: 120 - protein, 107 aa, 人源化
  10E11
EIVMTQSPATLSVSPGERATLSCRASQSVNNYLHWYQQKPGQAPRLLISYASQSISGIPARFSGSGSGTEFTLTISSLQSEDFAVYYCQQSNRWPLTFGQGTKLEIK

SEQ ID NO: 121 - protein, 445 aa, 人源化
  4E4
QVQLVQSGAEVKKPGASVKVSCKASGYTFTDHYMNWVRQAPGQGLEWIGDIDPKNGGTLYNQNFKGRATLTVDKSISTAYMELSRLRSDDTAVYYCARREAMDYWGQGTLVTVSSASTKGPSVFPLAPSSKSTSGGTAALGCLVKDYFPEPVTVSWNSGALTSGVHTFPAVLQSSGLYSLSSVVTVPSSSLGTQTYICNVNHKPSNTKVDKRVEPKSCDKTHTCPPCPAPELLGGPSVFLFPPKPKDTLMISRTPEVTCVVVDVSHEDPEVKFNWYVDGVEVHNAKTKPREEQYNSTYRVVSVLTVLHQDWLNGKEYKCKVSNKALPAPIEKTISKAKGQPREPQVYTLPPSRDELTKNQVSLTCLVKGFYPSDIAVEWESNGQPENNYKTTPPVLDSDGSFFLYSKLTVDKSRWQQGNVFSCSVMHEALHNHYTQKSLSLSPGK

SEQ ID NO: 122 - protein, 219 aa, 人源化
  4E4
DVVMTQSPLSLPVTPGEPASISCRSSQSIVYSNGNTYLNWYLQKPGQSPQLLIYKVSNRFSGVPDRFSGSGSGTDFTLKISRVEAEDVGVYYCFQGSHVPWTFGGGTKVEIKRTVAAPSVFIFPPSDEQLKSGTASVVCLLNNFYPREAKVQWKVDNALQSGNSQESVTEQDSKDSTYSLSSTLTLSKADYEKHKVYACEVTHQGLSSPVTKSFNRGEC

SEQ ID NO: 123 - protein, 449 aa, 人源化
  4B11
EVQLVQSGAEVKKPGASVKVSCKASGFTFTDSVLHWVRQAPGQRLEWIGYIHPYNDDTKFHDSFKGRATLTSDKSASTAYMELSSLRSEDTAVYYCSRNDELRVALDYWGQGTLVTVSSASTKGPSVFPLAPSSKSTSGGTAALGCLVKDYFPEPVTVSWNSGALTSGVHTFPAVLQSSGLYSLSSVVTVPSSSLGTQTYICNVNHKPSNTKVDKRVEPKSCDKTHTCPPCPAPELLGGPSVFLFPPKPKDTLMISRTPEVTCVVVDVSHEDPEVKFNWYVDGVEVHNAKTKPREEQYNSTYRVVSVLTVLHQDWLNGKEYKCKVSNKALPAPIEKTISKAKGQPREPQVYTLPPSRDELTKNQVSLTCLVKGFYPSDIAVEWESNGQPENNYKTTPPVLDSDGSFFLYSKLTVDKSRWQQGNVFSCSVMHEALHNHYTQKSLSLSPGK

SEQ ID NO: 124 - protein, 218 aa, 人源化
  4B11
EIVLTQSPATLSLSPGERATLSCRASQSVSTSTYSYVHWYQQKPGQAPRLLIKYASNLESGIPARFSGSGSGTDFTLTISSLEPEDFAVYYCQHSWGNPWTFGGGTKVEIKRTVAAPSVFIFPPSDEQLKSGTASVVCLLNNFYPREAKVQWKVDNALQSGNSQESVTEQDSKDSTYSLSSTLTLSKADYEKHKVYACEVTHQGLSSPVTKSFNRGEC

SEQ ID NO: 125 - protein, 442 aa, 人源化
  3F5
QVQLVQSGAEVKKPGASVKVSCKASGYTFTDHYMHWVRQAPGQGLEWIGDINPNSGGTINNQNFKGRATLTVDKSISTAYMELSRLRSDDTAVYYCARGFSGLAYWGQGTLVTVSSASTKGPSVFPLAPCSRSTSESTAALGCLVKDYFPEPVTVSWNSGALTSGVHTFPAVLQSSGLYSLSSVVTVPSSSLGTKTYTCNVDHKPSNTKVDKRVESKYGPPCPPCPAPEFLGGPSVFLFPPKPKDTLMISRTPEVTCVVVDVSQEDPEVQFNWYVDGVEVHNAKTKPREEQFNSTYRVVSVLTVLHQDWLNGKEYKCKVSNKGLPSSIEKTISKAKGQPREPQVYTLPPSQEEMTKNQVSLTCLVKGFYPSDIAVEWESNGQPENNYKTTPPVLDSDGSFFLYSRLTVDKSRWQEGNVFSCSVMHEALHNHYTQKSLSLSLG

SEQ ID NO: 126 - protein, 219 aa, 人源化
  3F5
DIVMTQTPLSSPVTLGQPASISCKSSQSLLDRDGKTYLNWLQQRPGQPPRRLIYLVSILDSGVPDRFSGSGAGTDFTLKISRVEAEDVGVYYCWQGTHFPWTFGQGTKLEIKRTVAAPSVFIFPPSDEQLKSGTASVVCLLNNFYPREAKVQWKVDNALQSGNSQESVTEQDSKDSTYSLSSTLTLSKADYEKHKVYACEVTHQGLSSPVTKSFNRGEC

SEQ ID NO: 127 - protein, 448 aa, 人源化
  10E11
EVQLVQSGAEVKKPGESLRISCKGSGYPVSRYWIEWVRQMPGKGLEWIGEILPGSDYANYNEKFKGHATFSADISISTAYLQWSSLKASDTAMYYCSRKGAYYALDFWGQGTLVTVSSASTKGPSVFPLAPSSKSTSGGTAALGCLVKDYFPEPVTVSWNSGALTSGVHTFPAVLQSSGLYSLSSVVTVPSSSLGTQTYICNVNHKPSNTKVDKRVEPKSCDKTHTCPPCPAPELLGGPSVFLFPPKPKDTLMISRTPEVTCVVVDVSHEDPEVKFNWYVDGVEVHNAKTKPREEQYNSTYRVVSVLTVLHQDWLNGKEYKCKVSNKALPAPIEKTISKAKGQPREPQVYTLPPSRDELTKNQVSLTCLVKGFYPSDIAVEWESNGQPENNYKTTPPVLDSDGSFFLYSKLTVDKSRWQQGNVFSCSVMHEALHNHYTQKSLSLSPGK

SEQ ID NO: 128 - protein, 448 aa, 人源化
  10E11
EVQLVQSGAEVKKPGESLRISCKASGYPVSRYWIEWVRQMPGKGLEWIGEILPGSDYANYNEKFKGHVTFSADISISTAYLQWSSLKASDTAMYYCSRKGAYYALDFWGQGTLVTVSSASTKGPSVFPLAPSSKSTSGGTAALGCLVKDYFPEPVTVSWNSGALTSGVHTFPAVLQSSGLYSLSSVVTVPSSSLGTQTYICNVNHKPSNTKVDKRVEPKSCDKTHTCPPCPAPELLGGPSVFLFPPKPKDTLMISRTPEVTCVVVDVSHEDPEVKFNWYVDGVEVHNAKTKPREEQYNSTYRVVSVLTVLHQDWLNGKEYKCKVSNKALPAPIEKTISKAKGQPREPQVYTLPPSRDELTKNQVSLTCLVKGFYPSDIAVEWESNGQPENNYKTTPPVLDSDGSFFLYSKLTVDKSRWQQGNVFSCSVMHEALHNHYTQKSLSLSPGK

SEQ ID NO: 129 - protein, 447 aa, 人源化
  10E11
EVQLVQSGAEVKKPGESLRISCKASGYPVSRYWIEWVRQMPGKGLEWIGEILPGSDYANYNEKFKGHVTFSADISISTAYLQWSSLKASDTAMYYCSRKGAYYALDFWGQGTLVTVSSASTKGPSVFPLAPSSKSTSGGTAALGCLVKDYFPEPVTVSWNSGALTSGVHTFPAVLQSSGLYSLSSVVTVPSSSLGTQTYICNVNHKPSNTKVDKKVEPKSCDKTHTCPPCPAPELLGGPSVFLFPPKPKDTLMISRTPEVTCVVVDVSHEDPEVKFNWYVDGVEVHNAKTKPREEQYNATYRVVSVLTVLHQDWLNGKEYKCKVSNKALPAPIAATISKAKGQPREPQVYTLPPSRDELTKNQVSLTCLVKGFYPSDIAVEWESNGQPENNYKTTPPVLDSDGSFFLYSKLTVDKSRWQQGNVFSCSVMHEALHNHYTQKSLSLSPG

SEQ ID NO: 130 - protein, 444 aa, 人源化
  10E11
EVQLVQSGAEVKKPGESLRISCKASGYPVSRYWIEWVRQMPGKGLEWIGEILPGSDYANYNEKFKGHVTFSADISISTAYLQWSSLKASDTAMYYCSRKGAYYALDFWGQGTLVTVSSASTKGPSVFPLAPCSRSTSESTAALGCLVKDYFPEPVTVSWNSGALTSGVHTFPAVLQSSGLYSLSSVVTVPSSSLGTKTYTCNVDHKPSNTKVDKRVESKYGPPCPPCPAPEFLGGPSVFLFPPKPKDTLMISRTPEVTCVVVDVSQEDPEVQFNWYVDGVEVHNAKTKPREEQFNSTYRVVSVLTVLHQDWLNGKEYKCKVSNKGLPSSIEKTISKAKGQPREPQVYTLPPSQEEMTKNQVSLTCLVKGFYPSDIAVEWESNGQPENNYKTTPPVLDSDGSFFLYSRLTVDKSRWQEGNVFSCSVMHEALHNHYTQKSLSLSLG

SEQ ID NO: 131 - protein, 214 aa, 人源化
  10E11
EIVMTQSPATLSVSPGERATLSCRASQSVNNYLHWYQQKPGQAPRLLISYASQSISGIPARFSGSGSGTEFTLTISSLQSEDFAVYYCQQSNRWPLTFGQGTKLEIKRTVAAPSVFIFPPSDEQLKSGTASVVCLLNNFYPREAKVQWKVDNALQSGNSQESVTEQDSKDSTYSLSSTLTLSKADYEKHKVYACEVTHQGLSSPVTKSFNRGEC